European Patent Application EP 4 296 284 A1, published December 27, 2023. Title: Bispecific single domain antibodies against PD-L1 and CD47 and use thereof. Applicant: SNU R&DB Foundation Shaperon. The sequence listing filed with the application follows.

SEQUENCE LISTING (22 sequences)

SEQ ID NO: 1 - protein, 120 aa, Artificial Sequence
  PDL1 Nb#01
QVQLVESGGGLVQPGGSLRLSCAASGFTFSSFAMSWVRQAPGKGLEWVSDINTGGDSTDYADSVKGRFTISRDNAKNTLYLQMNSLKPEDTAVYYCAKGPKEMVHVYSQRGQGTQVTVSS

SEQ ID NO: 2 - protein, 8 aa, Artificial Sequence
  PDL1 Nb#01_CDR1
GFTFSSFA

SEQ ID NO: 3 - protein, 8 aa, Artificial Sequence
  PDL1 Nb#01_CDR2
INTGGDST

SEQ ID NO: 4 - protein, 13 aa, Artificial Sequence
  PDL1 Nb#01_CDR3
AKGPKEMVHVYSQ

SEQ ID NO: 5 - protein, 357 aa, Artificial Sequence
  PDL1Nb#01-IgG1
QVQLVESGGGLVQPGGSLRLSCAASGFTFSSFAMSWVRQAPGKGLEWVSDINTGGDSTDYADSVKGRFTISRDNAKNTLYLQMNSLKPEDTAVYYCAKGPKEMVHVYSQRGQGTQVTVSSGPGGPEPKSSDKTHTCPPCPAPELLGGPSVFLFPPKPKDTLMISRTPEVTCVVVDVSHEDPEVKFNWYVDGVEVHNAKTKPREEQYNSTYRVVSVLTVLHQDWLNGKEYKCKVSNKALPAPIEKTISKAKGQPREPQVYTLPPSRDELTKNQVSLTCLVKGFYPSDIAVEWESNGQPENNYKTTPPVLDSDGSFFLYSKLTVDKSRWQQGNVFSCSVMHEALHNHYTQKSLSLSPGK

SEQ ID NO: 6 - protein, 123 aa, Artificial Sequence
  CD47 Nb#01
QVQLVESGGGLVQPGGSLNLSCAVSGLTFFRKYAVGWARQVPGKGLERVSRIYSDRRIEYLDAVKGRFTISRDNAKNTVYLQMNSLKTEDTAVYYCATGLRVGLTGWDEYDYWGQGTQVTVSS

SEQ ID NO: 7 - protein, 9 aa, Artificial Sequence
  CD47 Nb#01_CDR1
GLTFFRKYA

SEQ ID NO: 8 - protein, 7 aa, Artificial Sequence
  CD47 Nb#01_CDR2
IYSDRRI

SEQ ID NO: 9 - protein, 16 aa, Artificial Sequence
  CD47 Nb#01_CDR3
ATGLRVGLTGWDEYDY

SEQ ID NO: 10 - protein, 357 aa, Artificial Sequence
  CD47 Nb-IgG4
QVQLVESGGGLVQPGGSLNLSCAVSGLTFFRKYAVGWARQVPGKGLERVSRIYSDRRIEYLDAVKGRFTISRDNAKNTVYLQMNSLKTEDTAVYYCATGLRVGLTGWDEYDYWGQGTQVTVSSGPGGPESKYGPPCPPCPAPEFLGGPSVFLFPPKPKDTLMISRTPEVTCVVVDVSQEDPEVQFNWYVDGVEVHNAKTKPREEQFNSTYRVVSVLTVLHQDWLNGKEYKCKVSNKGLPSSIEKTISKAKGQPREPQVYTLPPSQEEMTKNQVSLTCLVKGFYPSDIAVEWESNGQPENNYKTTPPVLDSDGSFFLYSRLTVDKSRWQEGNVFSCSVMHEALHNHYTQKSLSLSPGK

SEQ ID NO: 11 - protein, 380 aa, Artificial Sequence
  PPC Nb
QVQLVESGGGLVQPGGSLRLSCAASGFTFSSFAMSWVRQAPGKGLEWVSDINTGGDSTDYADSVKGRFTISRDNAKNTLYLQMNSLKPEDTAVYYCAKGPKEMVHVYSQRGQGTQVTVSSGGSGGGPSQVQLVESGGGLVQPGGSLRLSCAASGFTFSSFAMSWVRQAPGKGLEWVSDINTGGDSTDYADSVKGRFTISRDNAKNTLYLQMNSLKPEDTAVYYCAKGPKEMVHVYSQRGQGTQVTVSSGGSGGSGGSQVQLVESGGGLVQPGGSLNLSCAVSGLTFFRKYAVGWARQVPGKGLERVSRIYSDRRIEYLDAVKGRFTISRDNAKNTVYLQMNSLKTEDTAVYYCATGLRVGLTGWDEYDYWGQGTQVTVSS

SEQ ID NO: 12 - protein, 734 aa, Artificial Sequence
  PPC Nb-IgG4
QVQLVESGGGLVQPGGSLRLSCAASGFTFSSFAMSWVRQAPGKGLEWVSDINTGGDSTDYADSVKGRFTISRDNAKNTLYLQMNSLKPEDTAVYYCAKGPKEMVHVYSQRGQGTQVTVSSQVQLVESGGGLVQPGGSLRLSCAASGFTFSSFAMSWVRQAPGKGLEWVSDINTGGDSTDYADSVKGRFTISRDNAKNTLYLQMNSLKPEDTAVYYCAKGPKEMVHVYSQRGQGTQVTVSSGGSGGGPSQVQLVESGGGLVQPGGSLRLSCAASGFTFSSFAMSWVRQAPGKGLEWVSDINTGGDSTDYADSVKGRFTISRDNAKNTLYLQMNSLKPEDTAVYYCAKGPKEMVHVYSQRGQGTQVTVSSGGSGGSGGSQVQLVESGGGLVQPGGSLNLSCAVSGLTFFRKYAVGWARQVPGKGLERVSRIYSDRRIEYLDAVKGRFTISRDNAKNTVYLQMNSLKTEDTAVYYCATGLRVGLTGWDEYDYWGQGTQVTVSSGPGGPESKYGPPCPPCPAPEFLGGPSVFLFPPKPKDTLMISRTPEVTCVVVDVSQEDPEVQFNWYVDGVEVHNAKTKPREEQFNSTYRVVSVLTVLHQDWLNGKEYKCKVSNKGLPSSIEKTISKAKGQPREPQVYTLPPSQEEMTKNQVSLTCLVKGFYPSDIAVEWESNGQPENNYKTTPPVLDSDGSFFLYSRLTVDKSRWQEGNVFSCSVMHEALHNHYTQKSLSLSPGK

SEQ ID NO: 13 - protein, 25 aa, Artificial Sequence
  PDL1 Nb#01_FR1
QVQLVESGGGLVQPGGSLRLSCAAS

SEQ ID NO: 14 - protein, 17 aa, Artificial Sequence
  PDL1 Nb#01_FR2
MSWVRQAPGKGLEWVSD

SEQ ID NO: 15 - protein, 38 aa, Artificial Sequence
  PDL1 Nb#01_FR3
DYADSVKGRFTISRDNAKNTLYLQMNSLKPEDTAVYYC

SEQ ID NO: 16 - protein, 11 aa, Artificial Sequence
  PDL1 Nb#01_FR4
RGQGTQVTVSS

SEQ ID NO: 17 - protein, 25 aa, Artificial Sequence
  CD47 Nb#01_FR1
QVQLVESGGGLVQPGGSLNLSCAVS

SEQ ID NO: 18 - protein, 17 aa, Artificial Sequence
  CD47 Nb#01_FR2
VGWARQVPGKGLERVSR

SEQ ID NO: 19 - protein, 38 aa, Artificial Sequence
  CD47 Nb#01_FR3
EYLDAVKGRFTISRDNAKNTVYLQMNSLKTEDTAVYYC

SEQ ID NO: 20 - protein, 11 aa, Artificial Sequence
  CD47 Nb#01_FR4
WGQGTQVTVSS

SEQ ID NO: 21 - protein, 246 aa, Artificial Sequence
  PP Nb
QVQLVESGGGLVQPGGSLRLSCAASGFTFSSFAMSWVRQAPGKGLEWVSDINTGGDSTDYADSVKGRFTISRDNAKNTLYLQMNSLKPEDTAVYYCAKGPKEMVHVYSQRGQGTQVTVSSGGSGGSQVQLVESGGGLVQPGGSLRLSCAASGFTFSSFAMSWVRQAPGKGLEWVSDINTGGDSTDYADSVKGRFTISRDNAKNTLYLQMNSLKPEDTAVYYCAKGPKEMVHVYSQRGQGTQVTVSS

SEQ ID NO: 22 - protein, 480 aa, Artificial Sequence
  PP Nb-IgG4
QVQLVESGGGLVQPGGSLRLSCAASGFTFSSFAMSWVRQAPGKGLEWVSDINTGGDSTDYADSVKGRFTISRDNAKNTLYLQMNSLKPEDTAVYYCAKGPKEMVHVYSQRGQGTQVTVSSGGSGGSQVQLVESGGGLVQPGGSLRLSCAASGFTFSSFAMSWVRQAPGKGLEWVSDINTGGDSTDYADSVKGRFTISRDNAKNTLYLQMNSLKPEDTAVYYCAKGPKEMVHVYSQRGQGTQVTVSSGPGGPESKYGPPCPPCPAPEFLGGPSVFLFPPKPKDTLMISRTPEVTCVVVDVSQEDPEVQFNWYVDGVEVHNAKTKPREEQFNSTYRVVSVLTVLHQDWLNGKEYKCKVSNKGLPSSIEKTISKAKGQPREPQVYTLPPSQEEMTKNQVSLTCLVKGFYPSDIAVEWESNGQPENNYKTTPPVLDSDGSFFLYSRLTVDKSRWQEGNVFSCSVMHEALHNHYTQKSLSLSPGK